European Patent Specification EP 4 188 371 B1, published September 2, 2026. Title: PRODUCTS FOR TREATING THE JNCL DISEASE. Applicant: BEYOND BATTEN DISEASE FOUNDATION BAYLOR COLLEGE OF MEDECINE UNIVERSITY COLLEGE CARDIFF CONSULTANTS LIMITED. The sequence listing filed with the application follows.

SEQUENCE LISTING (1 sequence)

SEQ ID NO: 1 - DNA, 25 bp, artificial
  cln3ATG morpholino
cattgcgactttcacaggagaaatg